European Patent Application EP 4 696 306 A1, published February 18, 2026. Title: Adenosine triphosphate secretion inhibitor, hepatic stellate cell activation inhibitor, hepatic stellate cell deactivator, liver fibrosis treatment agent, non-alcoholic steatohepatitis treatment agent, psoriasis treatment agent, and use of compound for manufacture of adenosine triphosphate secretion inhibitor, hepatic stellate cell activation inhibitor, hepatic stellate cell deactivator, liver fibrosis treatment agent, non-alcoholic steatohepatitis treatment agent and psoriasis treatment agent. Applicant: Kurume University. Application WO. The sequence listing filed with the application follows.

SEQUENCE LISTING (2 sequences)

SEQ ID NO: 1 - RNA, 22 nt, synthetic construct
  source 1..22: mol_type = other RNA
  modified_base 21: mod_base = OTHER; note = thymine
ctcatgaccttcacgcatcctc

SEQ ID NO: 2 - RNA, 26 nt, synthetic construct
  source 1..26: mol_type = other RNA
cggaagtactggaagagtgcgtagag